European Patent Specification EP 4 081 661 B1, published October 9, 2024. Title: MULTIPLEX DROP-OFF DIGITAL POLYMERASE CHAIN REACTION METHODS. Applicant: Stilla Technologies. Application Not Yet Assigned. The sequence listing filed with the application follows.

SEQUENCE LISTING (12 sequences)

SEQ ID NO: 1 - DNA, 26 bp, Artificial Sequence
  Synthetic Construct
tgaaaatgactgaatataaacttgtg

SEQ ID NO: 2 - DNA, 24 bp, Artificial Sequence
  Synthetic Construct
ctctattgttggatcatattcgtc

SEQ ID NO: 3 - DNA, 18 bp, Artificial Sequence
  Synthetic Construct
agtgccttgacgatacag

SEQ ID NO: 4 - DNA, 16 bp, Artificial Sequence
  Synthetic Construct
cctacgccaccagctc

SEQ ID NO: 5 - DNA, 23 bp, Artificial Sequence
  Synthetic Construct
caagtggttatagatggtgaaac

SEQ ID NO: 6 - DNA, 17 bp, Artificial Sequence
  Synthetic Construct
ccttcgcctgtcctcat

SEQ ID NO: 7 - DNA, 20 bp, Artificial Sequence
  Synthetic Construct
tttgttggacatactggata

SEQ ID NO: 8 - DNA, 18 bp, Artificial Sequence
  Synthetic Construct
  modified_base 3: Locked Nucleic Acid (LNA) base
  modified_base 6: Locked Nucleic Acid (LNA) base
  modified_base 11: Locked Nucleic Acid (LNA) base
agctggacaagaagagta

SEQ ID NO: 9 - DNA, 21 bp, Artificial Sequence
  Synthetic Construct
gtgagaaagttaaaattcccg

SEQ ID NO: 10 - DNA, 19 bp, Artificial Sequence
  Synthetic Construct
cacacagcaaagcagaaac

SEQ ID NO: 11 - DNA, 24 bp, Artificial Sequence
  Synthetic Construct
cacatcgaggatttccttgttggc

SEQ ID NO: 12 - DNA, 22 bp, Artificial Sequence
  Synthetic Construct
  modified_base 9: Locked Nucleic Acid (LNA) base
  modified_base 12: Locked Nucleic Acid (LNA) base
  modified_base 16: Locked Nucleic Acid (LNA) base
aggaattaagagaagcaacatc